European Patent Application EP 4 613 774 A1, published September 10, 2025. Title: SINGLE DOMAIN ANTIBODY TARGETING HUMAN ROR1. Applicant: Nanjing Probio Biotech Co., Ltd. Application CN. The sequence listing filed with the application follows.

SEQUENCE LISTING (90 sequences)

SEQ ID NO: 1 - protein, 120 aa, synthetic construct
EVQLVESGGGLAQAGGSLSLSCTASGRSFSNFQMGWFRQAPGKEREFVAASGWSGGPTYYADSVKGRFTISTDDSKKTMYLQMNSLKPEDTAAYYCYEDRVLSGRPVRYWGRGTQVTVSS

SEQ ID NO: 2 - protein, 8 aa, synthetic construct
GRSFSNFQ

SEQ ID NO: 3 - protein, 8 aa, synthetic construct
SGWSGGPT

SEQ ID NO: 4 - protein, 13 aa, synthetic construct
YEDRVLSGRPVRY

SEQ ID NO: 5 - DNA, 360 bp, synthetic construct
  source 1..360: mol_type = other DNA
gaagtgcagctggtggaaagcggcggcggcctggcgcaggcgggcggcagcctgagcctgagctgcaccgcgagcggccgtagctttagcaactttcagatgggctggtttcgtcaggcgccgggcaaagaacgtgaatttgtggcggcgagcggctggagcggcggcccgacctattatgcggatagcgtgaaaggccgttttaccattagcaccgatgatagcaaaaaaaccatgtatctgcagatgaacagcctgaaaccggaagataccgcggcgtattattgctatgaagatcgtgtgctgagcggccgtccggtgcgttattggggccgtggcacccaggtgaccgtgagcagc

SEQ ID NO: 6 - protein, 118 aa, synthetic construct
AVQLVDSGGGSVQPGESLTLSCTGSARFLSNYGMGWYRQFPGKMREMVAYETNRGNKRYAESVKGRFRIARDAAKTTVYLEMNSLKPEDTAVYYCNAESSGWGRRNYWGQGTQVTVSS

SEQ ID NO: 7 - protein, 8 aa, synthetic construct
ARFLSNYG

SEQ ID NO: 8 - protein, 7 aa, synthetic construct
ETNRGNK

SEQ ID NO: 9 - protein, 12 aa, synthetic construct
NAESSGWGRRNY

SEQ ID NO: 10 - DNA, 354 bp, synthetic construct
  source 1..354: mol_type = other DNA
gcggtgcagctggtggatagcggcggcggcagcgtgcagccgggcgaaagcctgaccctgagctgcaccggcagcgcgcgttttctgagcaactatggcatgggctggtatcgtcagtttccgggcaaaatgcgtgaaatggtggcgtatgaaaccaaccgtggcaacaaacgttatgcggaaagcgtgaaaggccgttttcgtattgcgcgtgatgcggcgaaaaccaccgtgtatctggaaatgaacagcctgaaaccggaagataccgcggtgtattattgcaacgcggaaagcagcggctggggccgtcgtaactattggggccagggcacccaggtgaccgtgagcagc

SEQ ID NO: 11 - protein, 111 aa, synthetic construct
QVQLVESGGGVVQPGGSLRLSCAASGFVLRVNTVSWYRQAPGKQRELVALITSESNEYYDDSVKGRFTISRDNAKNTIYLHMNSLKPEDTGVYFCNFITTWGQGTQVTVSS

SEQ ID NO: 12 - protein, 8 aa, synthetic construct
GFVLRVNT

SEQ ID NO: 13 - protein, 7 aa, synthetic construct
ITSESNE

SEQ ID NO: 14 - protein, 5 aa, synthetic construct
NFITT

SEQ ID NO: 15 - DNA, 333 bp, synthetic construct
  source 1..333: mol_type = other DNA
caggtgcagctggtggaaagcggcggcggcgtggtgcagccgggcggcagcctgcgtctgagctgcgcggcgagcggctttgtgctgcgtgtgaacaccgtgagctggtatcgtcaggcgccgggcaaacagcgtgaactggtggcgctgattaccagcgaaagcaacgaatattatgatgatagcgtgaaaggccgttttaccattagccgtgataacgcgaaaaacaccatttatctgcatatgaacagcctgaaaccggaagataccggcgtgtatttttgcaactttattaccacctggggccagggcacccaggtgaccgtgagcagc

SEQ ID NO: 16 - protein, 111 aa, synthetic construct
EVQLVESGGGLVQPGGTLRLSCAASGSISRFYAVGWYRQAPGKQRELVARISSGGSTYYADSVKGRFTISINNSKNTVYLQMNNLKPEDTAVYYCNARNLWGQGTQVTVSS

SEQ ID NO: 17 - protein, 8 aa, synthetic construct
GSISRFYA

SEQ ID NO: 18 - protein, 7 aa, synthetic construct
ISSGGST

SEQ ID NO: 19 - protein, 5 aa, synthetic construct
NARNL

SEQ ID NO: 20 - DNA, 333 bp, synthetic construct
  source 1..333: mol_type = other DNA
gaagtgcagctggtggaaagcggcggcggcctggtgcagccgggcggcaccctgcgtctgagctgcgcggcgagcggcagcattagccgtttttatgcggtgggctggtatcgtcaggcgccgggcaaacagcgtgaactggtggcgcgtattagcagcggcggcagcacctattatgcggatagcgtgaaaggccgttttaccattagcattaacaacagcaaaaacaccgtgtatctgcagatgaacaacctgaaaccggaagataccgcggtgtattattgcaacgcgcgtaacctgtggggccagggcacccaggtgaccgtgagcagc

SEQ ID NO: 21 - protein, 126 aa, synthetic construct
QVQLVESGGGSVQAGGSLRLSCAVSGRSISLYNMGWFRQAPGKEREFVSAINWSGGRTYYADSVKGRFTISRNNAKNTMYLQMNSLKPEDTATYYCAVDVEGWFRVSGDAAGYDYWGQGTQVTVSS

SEQ ID NO: 22 - protein, 8 aa, synthetic construct
GRSISLYN

SEQ ID NO: 23 - protein, 8 aa, synthetic construct
INWSGGRT

SEQ ID NO: 24 - protein, 19 aa, synthetic construct
AVDVEGWFRVSGDAAGYDY

SEQ ID NO: 25 - DNA, 378 bp, synthetic construct
  source 1..378: mol_type = other DNA
caggtgcagctggtggaaagcggcggcggcagcgtgcaggcgggcggcagcctgcgtctgagctgcgcggtgagcggccgtagcattagcctgtataacatgggctggtttcgtcaggcgccgggcaaagaacgtgaatttgtgagcgcgattaactggagcggcggccgtacctattatgcggatagcgtgaaaggccgttttaccattagccgtaacaacgcgaaaaacaccatgtatctgcagatgaacagcctgaaaccggaagataccgcgacctattattgcgcggtggatgtggaaggctggtttcgtgtgagcggcgatgcggcgggctatgattattggggccagggcacccaggtgaccgtgagcagc

SEQ ID NO: 26 - protein, 119 aa, synthetic construct
EVQLVESGGGLVQPGGSLRLSCLASGSDFSDSAMGWYRQAPGKQREFVAAIGAGGITTYADSVKGRFTISRDSAKNIVYLQMSSLSPEDTAVYFCNFAPGWYPPGYQYWGQGTQVTVSS

SEQ ID NO: 27 - protein, 8 aa, synthetic construct
GSDFSDSA

SEQ ID NO: 28 - protein, 7 aa, synthetic construct
IGAGGIT

SEQ ID NO: 29 - protein, 13 aa, synthetic construct
NFAPGWYPPGYQY

SEQ ID NO: 30 - DNA, 357 bp, synthetic construct
  source 1..357: mol_type = other DNA
gaagtgcagctggtggaaagcggcggcggcctggtgcagccgggcggcagcctgcgtctgagctgcctggcgagcggcagcgattttagcgatagcgcgatgggctggtatcgtcaggcgccgggcaaacagcgtgaatttgtggcggcgattggcgcgggcggcattaccacctatgcggatagcgtgaaaggccgttttaccattagccgtgatagcgcgaaaaacattgtgtatctgcagatgagcagcctgagcccggaagataccgcggtgtatttttgcaactttgcgccgggctggtatccgccgggctatcagtattggggccagggcacccaggtgaccgtgagcagc

SEQ ID NO: 31 - protein, 121 aa, synthetic construct
QVQLVESGGGLVQPGGSLTLSCAASQSISSIYLLGWYRQAPGKERESVARITTSGTTTYIADSVKGRFTLSRDNAKNTMYLQMNSLKPEDTAVYYCNVPFLVATARGNAYWGQGTQVTVSS

SEQ ID NO: 32 - protein, 8 aa, synthetic construct
QSISSIYL

SEQ ID NO: 33 - protein, 8 aa, synthetic construct
ITTSGTTT

SEQ ID NO: 34 - protein, 14 aa, synthetic construct
NVPFLVATARGNAY

SEQ ID NO: 35 - DNA, 363 bp, synthetic construct
  source 1..363: mol_type = other DNA
caggtgcagctggtggaaagcggcggcggcctggtgcagccgggcggcagcctgaccctgagctgcgcggcgagccagagcattagcagcatttatctgctgggctggtatcgtcaggcgccgggcaaagaacgtgaaagcgtggcgcgtattaccaccagcggcaccaccacctatattgcggatagcgtgaaaggccgttttaccctgagccgtgataacgcgaaaaacaccatgtatctgcagatgaacagcctgaaaccggaagataccgcggtgtattattgcaacgtgccgtttctggtggcgaccgcgcgtggcaacgcgtattggggccagggcacccaggtgaccgtgagcagc

SEQ ID NO: 36 - protein, 115 aa, synthetic construct
QVQLVESGGGLVQPGGSLRLSCAVLGSIEQINDINYYRWYRQPPGKQRDLVASINNSGELIYADSVKGRFFISRDKYTVYLEMRSLKAEDTAVYYCNAQDRGEYWGRGTQVTVSS

SEQ ID NO: 37 - protein, 8 aa, synthetic construct
GSIEQIND

SEQ ID NO: 38 - protein, 8 aa, synthetic construct
VASINNSG

SEQ ID NO: 39 - protein, 8 aa, synthetic construct
NAQDRGEY

SEQ ID NO: 40 - DNA, 345 bp, synthetic construct
  source 1..345: mol_type = other DNA
caggtgcagctggtggaaagcggcggcggcctggtgcagccgggcggcagcctgcgtctgagctgcgcggtgctgggcagcattgaacagattaacgatattaactattatcgttggtatcgtcagccgccgggcaaacagcgtgatctggtggcgagcattaacaacagcggcgaactgatttatgcggatagcgtgaaaggccgtttttttattagccgtgataaatataccgtgtatctggaaatgcgtagcctgaaagcggaagataccgcggtgtattattgcaacgcgcaggatcgtggcgaatattggggccgtggcacccaggtgaccgtgagcagc

SEQ ID NO: 41 - protein, 120 aa, synthetic construct
EVQLVESGGGLVQPGGSLRLSCAASGRSFSNFQMGWFRQAPGKEREFVAASGWSGGPTYYADSVKGRFTISTDNSKNTLYLQMNSLRAEDTAVYYCYEDRVLSGRPVRYWGQGTLVTVSS

SEQ ID NO: 42 - DNA, 360 bp, synthetic construct
  source 1..360: mol_type = other DNA
gaagtgcagctggtcgagagcggcggcggcctggttcaacctggaggatctctgagactgtcttgtgctgcttctggcagaagcttcagcaacttccagatgggctggtttagacaggcccctggcaaagagcgggaattcgtggccgccagcggctggtccggcggaccaacatactatgccgacagcgtgaagggcagattcacaatcagcaccgacaatagcaagaacaccctgtacctgcagatgaacagcctgcgggccgaggacaccgccgtgtactactgctacgaggatagagtgctgagcggccgccccgtgcggtactggggccagggcaccctcgtgaccgtgtccagc

SEQ ID NO: 43 - protein, 111 aa, synthetic construct
EVQLVESGGGLVQPGGSLRLSCAASGSISRFYAVGWYRQAPGKQRELVARISSGGSTYYADSVKGRFTISIDNSKNTLYLQMNSLRAEDTAVYYCNARNLWGQGTLVTVSS

SEQ ID NO: 44 - DNA, 333 bp, synthetic construct
  source 1..333: mol_type = other DNA
gaagtgcaactggtcgagagcggcggaggactggtgcagcccggcggctctctgagactgagctgcgccgctagcggcagcatctctagattctacgccgtgggctggtatagacaggcccctggcaaacagcgggaactggtggccagaatcagctctggcggaagcacctactacgctgatagcgtgaagggcagattcaccatctccatcgacaacagcaagaacaccctctacctgcagatgaacagcctgcgggccgaggacaccgccgtgtactactgtaatgcccggaacctgtggggccagggcacactggttacagtgtccagc

SEQ ID NO: 45 - protein, 119 aa, synthetic construct
EVQLVESGGGLVQPGGSLRLSCAASGSDFSDSAMGWYRQAPGKQREFVAAIGAGGITTYADSVKGRFTISRDNAKNTLYLQMNSLRAEDTAVYFCNFAPGWYPPGYQYWGQGTLVTVSS

SEQ ID NO: 46 - DNA, 357 bp, synthetic construct
  source 1..357: mol_type = other DNA
gaagtgcagctggtggaaagcggcggaggactggtccaacctggcggatctctgagactgagctgcgccgcttctggctccgatttcagcgacagcgccatgggctggtacagacaggcccctggcaaacagagagagttcgtggctgctatcggcgccggcggcatcaccacctacgccgatagcgtgaagggcagattcacaatcagccgggacaacgccaagaacaccctgtacctgcagatgaacagcctgcgggccgaggacaccgccgtgtacttttgtaatttcgcccccggctggtatcctccaggataccagtactggggccagggcacactcgtgaccgtgtccagc

SEQ ID NO: 47 - protein, 937 aa, Homo sapiens
MHRPRRRGTRPPLLALLAALLLAARGAAAQETELSVSAELVPTSSWNISSELNKDSYLTLDEPMNNITTSLGQTAELHCKVSGNPPPTIRWFKNDAPVVQEPRRLSFRSTIYGSRLRIRNLDTTDTGYFQCVATNGKEVVSSTGVLFVKFGPPPTASPGYSDEYEEDGFCQPYRGIACARFIGNRTVYMESLHMQGEIENQITAAFTMIGTSSHLSDKCSQFAIPSLCHYAFPYCDETSSVPKPRDLCRDECEILENVLCQTEYIFARSNPMILMRLKLPNCEDLPQPESPEAANCIRIGIPMADPINKNHKCYNSTGVDYRGTVSVTKSGRQCQPWNSQYPHTHTFTALRFPELNGGHSYCRNPGNQKEAPWCFTLDENFKSDLCDIPACDSKDSKEKNKMEILYILVPSVAIPLAIALLFFFICVCRNNQKSSSAPVQRQPKHVRGQNVEMSMLNAYKPKSKAKELPLSAVRFMEELGECAFGKIYKGHLYLPGMDHAQLVAIKTLKDYNNPQQWTEFQQEASLMAELHHPNIVCLLGAVTQEQPVCMLFEYINQGDLHEFLIMRSPHSDVGCSSDEDGTVKSSLDHGDFLHIAIQIAAGMEYLSSHFFVHKDLAARNILIGEQLHVKISDLGLSREIYSADYYRVQSKSLLPIRWMPPEAIMYGKFSSDSDIWSFGVVLWEIFSFGLQPYYGFSNQEVIEMVRKRQLLPCSEDCPPRMYSLMTECWNEIPSRRPRFKDIHVRLRSWEGLSSHTSSTTPSGGNATTQTTSLSASPVSNLSNPRYPNYMFPSQGITPQGQIAGFIGPPIPQNQRFIPINGYPIPPGYAAFPAAHYQPTGPPRVIQHCPPPKSRSPSSASGSTSTGHVTSLPSSGSNQEANIPLLPHMSIPNHPGGMGITVFGNKSQKPYKIDSKQASLLGDANIHGHTESMISAEL

SEQ ID NO: 48 - protein, 22 aa, synthetic construct
MLLLVTSLLLCELPHPAFLLIP

SEQ ID NO: 49 - protein, 15 aa, synthetic construct
GGGGSGGGGSGGGGS

SEQ ID NO: 50 - protein, 12 aa, synthetic construct
ESKYGPPCPPCP

SEQ ID NO: 51 - protein, 27 aa, synthetic construct
FWVLVVVGGVLACYSLLVTVAFIIFWV

SEQ ID NO: 52 - protein, 42 aa, synthetic construct
KRGRKKLLYIFKQPFMRPVQTTQEEDGCSCRFPEEEEGGCEL

SEQ ID NO: 53 - protein, 112 aa, synthetic construct
RVKFSRSADAPAYQQGQNQLYNELNLGRREEYDVLDKRRGRDPEMGGKPRRKNPQEGLYNELQKDKMAEAYSEIGMKGERRRGKGHDGLYQGLSTATKDTYDALHMQALPPR

SEQ ID NO: 54 - protein, 24 aa, synthetic construct
LEGGGEGRGSLLTCGDVEENPGPR

SEQ ID NO: 55 - protein, 357 aa, synthetic construct
MLLLVTSLLLCELPHPAFLLIPRKVCNGIGIGEFKDSLSINATNIKHFKNCTSISGDLHILPVAFRGDSFTHTPPLDPQELDILKTVKEITGFLLIQAWPENRTDLHAFENLEIIRGRTKQHGQFSLAVVSLNITSLGLRSLKEISDGDVIISGNKNLCYANTINWKKLFGTSGQKTKIISNRGENSCKATGQVCHALCSPEGCWGPEPRDCVSCRNVSRGRECVDKCNLLEGEPREFVENSECIQCHPECLPQAMNITCTGRGPDNCIQCAHYIDGPHCVKTCPAGVMGENNTLVWKYADAGHVCHLCHPNCTYGCTGPGLEGCPTNGPKIPSIATGMVGALLLLLVVALGIGLFM

SEQ ID NO: 56 - protein, 716 aa, synthetic construct
MLLLVTSLLLCELPHPAFLLIPEVQLVESGGGLAQAGGSLSLSCTASGRSFSNFQMGWFRQAPGKEREFVAASGWSGGPTYYADSVKGRFTISTDDSKKTMYLQMNSLKPEDTAAYYCYEDRVLSGRPVRYWGRGTQVTVSSESKYGPPCPPCPFWVLVVVGGVLACYSLLVTVAFIIFWVKRGRKKLLYIFKQPFMRPVQTTQEEDGCSCRFPEEEEGGCELRVKFSRSADAPAYQQGQNQLYNELNLGRREEYDVLDKRRGRDPEMGGKPRRKNPQEGLYNELQKDKMAEAYSEIGMKGERRRGKGHDGLYQGLSTATKDTYDALHMQALPPRLEGGGEGRGSLLTCGDVEENPGPRMLLLVTSLLLCELPHPAFLLIPRKVCNGIGIGEFKDSLSINATNIKHFKNCTSISGDLHILPVAFRGDSFTHTPPLDPQELDILKTVKEITGFLLIQAWPENRTDLHAFENLEIIRGRTKQHGQFSLAVVSLNITSLGLRSLKEISDGDVIISGNKNLCYANTINWKKLFGTSGQKTKIISNRGENSCKATGQVCHALCSPEGCWGPEPRDCVSCRNVSRGRECVDKCNLLEGEPREFVENSECIQCHPECLPQAMNITCTGRGPDNCIQCAHYIDGPHCVKTCPAGVMGENNTLVWKYADAGHVCHLCHPNCTYGCTGPGLEGCPTNGPKIPSIATGMVGALLLLLVVALGIGLFM

SEQ ID NO: 57 - protein, 707 aa, synthetic construct
MLLLVTSLLLCELPHPAFLLIPQVQLVESGGGVVQPGGSLRLSCAASGFVLRVNTVSWYRQAPGKQRELVALITSESNEYYDDSVKGRFTISRDNAKNTIYLHMNSLKPEDTGVYFCNFITTWGQGTQVTVSSESKYGPPCPPCPFWVLVVVGGVLACYSLLVTVAFIIFWVKRGRKKLLYIFKQPFMRPVQTTQEEDGCSCRFPEEEEGGCELRVKFSRSADAPAYQQGQNQLYNELNLGRREEYDVLDKRRGRDPEMGGKPRRKNPQEGLYNELQKDKMAEAYSEIGMKGERRRGKGHDGLYQGLSTATKDTYDALHMQALPPRLEGGGEGRGSLLTCGDVEENPGPRMLLLVTSLLLCELPHPAFLLIPRKVCNGIGIGEFKDSLSINATNIKHFKNCTSISGDLHILPVAFRGDSFTHTPPLDPQELDILKTVKEITGFLLIQAWPENRTDLHAFENLEIIRGRTKQHGQFSLAVVSLNITSLGLRSLKEISDGDVIISGNKNLCYANTINWKKLFGTSGQKTKIISNRGENSCKATGQVCHALCSPEGCWGPEPRDCVSCRNVSRGRECVDKCNLLEGEPREFVENSECIQCHPECLPQAMNITCTGRGPDNCIQCAHYIDGPHCVKTCPAGVMGENNTLVWKYADAGHVCHLCHPNCTYGCTGPGLEGCPTNGPKIPSIATGMVGALLLLLVVALGIGLFM

SEQ ID NO: 58 - protein, 707 aa, synthetic construct
MLLLVTSLLLCELPHPAFLLIPEVQLVESGGGLVQPGGTLRLSCAASGSISRFYAVGWYRQAPGKQRELVARISSGGSTYYADSVKGRFTISINNSKNTVYLQMNNLKPEDTAVYYCNARNLWGQGTQVTVSSESKYGPPCPPCPFWVLVVVGGVLACYSLLVTVAFIIFWVKRGRKKLLYIFKQPFMRPVQTTQEEDGCSCRFPEEEEGGCELRVKFSRSADAPAYQQGQNQLYNELNLGRREEYDVLDKRRGRDPEMGGKPRRKNPQEGLYNELQKDKMAEAYSEIGMKGERRRGKGHDGLYQGLSTATKDTYDALHMQALPPRLEGGGEGRGSLLTCGDVEENPGPRMLLLVTSLLLCELPHPAFLLIPRKVCNGIGIGEFKDSLSINATNIKHFKNCTSISGDLHILPVAFRGDSFTHTPPLDPQELDILKTVKEITGFLLIQAWPENRTDLHAFENLEIIRGRTKQHGQFSLAVVSLNITSLGLRSLKEISDGDVIISGNKNLCYANTINWKKLFGTSGQKTKIISNRGENSCKATGQVCHALCSPEGCWGPEPRDCVSCRNVSRGRECVDKCNLLEGEPREFVENSECIQCHPECLPQAMNITCTGRGPDNCIQCAHYIDGPHCVKTCPAGVMGENNTLVWKYADAGHVCHLCHPNCTYGCTGPGLEGCPTNGPKIPSIATGMVGALLLLLVVALGIGLFM

SEQ ID NO: 59 - protein, 715 aa, synthetic construct
MLLLVTSLLLCELPHPAFLLIPEVQLVESGGGLVQPGGSLRLSCLASGSDFSDSAMGWYRQAPGKQREFVAAIGAGGITTYADSVKGRFTISRDSAKNIVYLQMSSLSPEDTAVYFCNFAPGWYPPGYQYWGQGTQVTVSSESKYGPPCPPCPFWVLVVVGGVLACYSLLVTVAFIIFWVKRGRKKLLYIFKQPFMRPVQTTQEEDGCSCRFPEEEEGGCELRVKFSRSADAPAYQQGQNQLYNELNLGRREEYDVLDKRRGRDPEMGGKPRRKNPQEGLYNELQKDKMAEAYSEIGMKGERRRGKGHDGLYQGLSTATKDTYDALHMQALPPRLEGGGEGRGSLLTCGDVEENPGPRMLLLVTSLLLCELPHPAFLLIPRKVCNGIGIGEFKDSLSINATNIKHFKNCTSISGDLHILPVAFRGDSFTHTPPLDPQELDILKTVKEITGFLLIQAWPENRTDLHAFENLEIIRGRTKQHGQFSLAVVSLNITSLGLRSLKEISDGDVIISGNKNLCYANTINWKKLFGTSGQKTKIISNRGENSCKATGQVCHALCSPEGCWGPEPRDCVSCRNVSRGRECVDKCNLLEGEPREFVENSECIQCHPECLPQAMNITCTGRGPDNCIQCAHYIDGPHCVKTCPAGVMGENNTLVWKYADAGHVCHLCHPNCTYGCTGPGLEGCPTNGPKIPSIATGMVGALLLLLVVALGIGLFM

SEQ ID NO: 60 - protein, 722 aa, synthetic construct
MLLLVTSLLLCELPHPAFLLIPQVQLVESGGGSVQAGGSLRLSCAVSGRSISLYNMGWFRQAPGKEREFVSAINWSGGRTYYADSVKGRFTISRNNAKNTMYLQMNSLKPEDTATYYCAVDVEGWFRVSGDAAGYDYWGQGTQVTVSSESKYGPPCPPCPFWVLVVVGGVLACYSLLVTVAFIIFWVKRGRKKLLYIFKQPFMRPVQTTQEEDGCSCRFPEEEEGGCELRVKFSRSADAPAYQQGQNQLYNELNLGRREEYDVLDKRRGRDPEMGGKPRRKNPQEGLYNELQKDKMAEAYSEIGMKGERRRGKGHDGLYQGLSTATKDTYDALHMQALPPRLEGGGEGRGSLLTCGDVEENPGPRMLLLVTSLLLCELPHPAFLLIPRKVCNGIGIGEFKDSLSINATNIKHFKNCTSISGDLHILPVAFRGDSFTHTPPLDPQELDILKTVKEITGFLLIQAWPENRTDLHAFENLEIIRGRTKQHGQFSLAVVSLNITSLGLRSLKEISDGDVIISGNKNLCYANTINWKKLFGTSGQKTKIISNRGENSCKATGQVCHALCSPEGCWGPEPRDCVSCRNVSRGRECVDKCNLLEGEPREFVENSECIQCHPECLPQAMNITCTGRGPDNCIQCAHYIDGPHCVKTCPAGVMGENNTLVWKYADAGHVCHLCHPNCTYGCTGPGLEGCPTNGPKIPSIATGMVGALLLLLVVALGIGLFM

SEQ ID NO: 61 - protein, 711 aa, synthetic construct
MLLLVTSLLLCELPHPAFLLIPQVQLVESGGGLVQPGGSLRLSCAVLGSIEQINDINYYRWYRQPPGKQRDLVASINNSGELIYADSVKGRFFISRDKYTVYLEMRSLKAEDTAVYYCNAQDRGEYWGRGTQVTVSSESKYGPPCPPCPFWVLVVVGGVLACYSLLVTVAFIIFWVKRGRKKLLYIFKQPFMRPVQTTQEEDGCSCRFPEEEEGGCELRVKFSRSADAPAYQQGQNQLYNELNLGRREEYDVLDKRRGRDPEMGGKPRRKNPQEGLYNELQKDKMAEAYSEIGMKGERRRGKGHDGLYQGLSTATKDTYDALHMQALPPRLEGGGEGRGSLLTCGDVEENPGPRMLLLVTSLLLCELPHPAFLLIPRKVCNGIGIGEFKDSLSINATNIKHFKNCTSISGDLHILPVAFRGDSFTHTPPLDPQELDILKTVKEITGFLLIQAWPENRTDLHAFENLEIIRGRTKQHGQFSLAVVSLNITSLGLRSLKEISDGDVIISGNKNLCYANTINWKKLFGTSGQKTKIISNRGENSCKATGQVCHALCSPEGCWGPEPRDCVSCRNVSRGRECVDKCNLLEGEPREFVENSECIQCHPECLPQAMNITCTGRGPDNCIQCAHYIDGPHCVKTCPAGVMGENNTLVWKYADAGHVCHLCHPNCTYGCTGPGLEGCPTNGPKIPSIATGMVGALLLLLVVALGIGLFM

SEQ ID NO: 62 - protein, 714 aa, synthetic construct
MLLLVTSLLLCELPHPAFLLIPAVQLVDSGGGSVQPGESLTLSCTGSARFLSNYGMGWYRQFPGKMREMVAYETNRGNKRYAESVKGRFRIARDAAKTTVYLEMNSLKPEDTAVYYCNAESSGWGRRNYWGQGTQVTVSSESKYGPPCPPCPFWVLVVVGGVLACYSLLVTVAFIIFWVKRGRKKLLYIFKQPFMRPVQTTQEEDGCSCRFPEEEEGGCELRVKFSRSADAPAYQQGQNQLYNELNLGRREEYDVLDKRRGRDPEMGGKPRRKNPQEGLYNELQKDKMAEAYSEIGMKGERRRGKGHDGLYQGLSTATKDTYDALHMQALPPRLEGGGEGRGSLLTCGDVEENPGPRMLLLVTSLLLCELPHPAFLLIPRKVCNGIGIGEFKDSLSINATNIKHFKNCTSISGDLHILPVAFRGDSFTHTPPLDPQELDILKTVKEITGFLLIQAWPENRTDLHAFENLEIIRGRTKQHGQFSLAVVSLNITSLGLRSLKEISDGDVIISGNKNLCYANTINWKKLFGTSGQKTKIISNRGENSCKATGQVCHALCSPEGCWGPEPRDCVSCRNVSRGRECVDKCNLLEGEPREFVENSECIQCHPECLPQAMNITCTGRGPDNCIQCAHYIDGPHCVKTCPAGVMGENNTLVWKYADAGHVCHLCHPNCTYGCTGPGLEGCPTNGPKIPSIATGMVGALLLLLVVALGIGLFM

SEQ ID NO: 63 - protein, 717 aa, synthetic construct
MLLLVTSLLLCELPHPAFLLIPQVQLVESGGGLVQPGGSLTLSCAASQSISSIYLLGWYRQAPGKERESVARITTSGTTTYIADSVKGRFTLSRDNAKNTMYLQMNSLKPEDTAVYYCNVPFLVATARGNAYWGQGTQVTVSSESKYGPPCPPCPFWVLVVVGGVLACYSLLVTVAFIIFWVKRGRKKLLYIFKQPFMRPVQTTQEEDGCSCRFPEEEEGGCELRVKFSRSADAPAYQQGQNQLYNELNLGRREEYDVLDKRRGRDPEMGGKPRRKNPQEGLYNELQKDKMAEAYSEIGMKGERRRGKGHDGLYQGLSTATKDTYDALHMQALPPRLEGGGEGRGSLLTCGDVEENPGPRMLLLVTSLLLCELPHPAFLLIPRKVCNGIGIGEFKDSLSINATNIKHFKNCTSISGDLHILPVAFRGDSFTHTPPLDPQELDILKTVKEITGFLLIQAWPENRTDLHAFENLEIIRGRTKQHGQFSLAVVSLNITSLGLRSLKEISDGDVIISGNKNLCYANTINWKKLFGTSGQKTKIISNRGENSCKATGQVCHALCSPEGCWGPEPRDCVSCRNVSRGRECVDKCNLLEGEPREFVENSECIQCHPECLPQAMNITCTGRGPDNCIQCAHYIDGPHCVKTCPAGVMGENNTLVWKYADAGHVCHLCHPNCTYGCTGPGLEGCPTNGPKIPSIATGMVGALLLLLVVALGIGLFM

SEQ ID NO: 64 - protein, 844 aa, synthetic construct
MLLLVTSLLLCELPHPAFLLIPQEQLVESGGRLVTPGGSLTLSCKASGFDFSAYYMSWVRQAPGKGLEWIATIYPSSGKTYYATWVNGRFTISSDNAQNTVDLQMNSLTAADRATYFCARDSYADDGALFNIWGPGTLVTISSGGGGSGGGGSGGGGSELVLTQSPSVSAALGSPAKITCTLSSAHKTDTIDWYQQLQGEAPRYLMQVQSDGSYTKRPGVPDRFSGSSSGADRYLIIPSVQADDEADYYCGADYIGGYVFGGGTQLTVTGESKYGPPCPPCPFWVLVVVGGVLACYSLLVTVAFIIFWVKRGRKKLLYIFKQPFMRPVQTTQEEDGCSCRFPEEEEGGCELRVKFSRSADAPAYQQGQNQLYNELNLGRREEYDVLDKRRGRDPEMGGKPRRKNPQEGLYNELQKDKMAEAYSEIGMKGERRRGKGHDGLYQGLSTATKDTYDALHMQALPPRLEGGGEGRGSLLTCGDVEENPGPRMLLLVTSLLLCELPHPAFLLIPRKVCNGIGIGEFKDSLSINATNIKHFKNCTSISGDLHILPVAFRGDSFTHTPPLDPQELDILKTVKEITGFLLIQAWPENRTDLHAFENLEIIRGRTKQHGQFSLAVVSLNITSLGLRSLKEISDGDVIISGNKNLCYANTINWKKLFGTSGQKTKIISNRGENSCKATGQVCHALCSPEGCWGPEPRDCVSCRNVSRGRECVDKCNLLEGEPREFVENSECIQCHPECLPQAMNITCTGRGPDNCIQCAHYIDGPHCVKTCPAGVMGENNTLVWKYADAGHVCHLCHPNCTYGCTGPGLEGCPTNGPKIPSIATGMVGALLLLLVVALGIGLFM

SEQ ID NO: 65 - protein, 120 aa, synthetic construct
EVQLVESGGGLVQPGGSLRLSCAASGRSFSSFQMGWFRQAPGKEREFVAASGWSGGPTYYWDSVIGRFTISTDNSKNTLYLQMNSLRAEDTAVYYCYEDRVLSGRHVRYWGQGTLVTVSS

SEQ ID NO: 66 - protein, 8 aa, synthetic construct
GRSFSSFQ

SEQ ID NO: 67 - protein, 13 aa, synthetic construct
YEDRVLSGRHVRY

SEQ ID NO: 68 - protein, 120 aa, synthetic construct
EVQLVESGGGLVQPGGSLRLSCAASGRSFSSFQMGWFRQAPGKEREFVAASGWSGGPTYYWDSWKGRFTISTDNSKNTLYLQMNSLRAEDTAVYYCYEDKVLSGRRVRYWGQGTLVTVSS

SEQ ID NO: 69 - protein, 13 aa, synthetic construct
YEDKVLSGRRVRY

SEQ ID NO: 70 - protein, 120 aa, synthetic construct
EVQLVESGGGLVQPGGSLRLSCAASGRSFSSFQMGWFRQAPGKEREFVAASGWSGGPTYYWDSWKGRFTISTDNSKNTLYLQMNSLRAEDTAVYYCYEDRVLSGRWVRYWGQGTLVTVSS

SEQ ID NO: 71 - protein, 13 aa, synthetic construct
YEDRVLSGRWVRY

SEQ ID NO: 72 - protein, 120 aa, synthetic construct
EVQLVESGGGLVQPGGSLRLSCAASGRSFSNFQMGWFRQAPGKEREFVAASGWSGGPTYYWDSVIGRFTISTDNSKNTLYLQMNSLRAEDTAVYYCYEDRVLSGRPVRYWGQGTLVTVSS

SEQ ID NO: 73 - protein, 120 aa, synthetic construct
EVQLVESGGGLVQPGGSLRLSCAASGRSFSSFQMGWFRQAPGKEREFVAASGWSGGPTYYWDSVIGRFTISTDNSKNTLYLQMNSLRAEDTAVYYCYEDRVLSGRPVRYWGQGTLVTVSS

SEQ ID NO: 74 - protein, 111 aa, synthetic construct
EVQLVESGGGLVQPGGSLRLSCAASYYISRFYAVGWYRQAPGKQRELVARISSGGWTYYADSVKGRFTISIDNSKNTLYLQMNSLRAEDTAVYYCNARNLWGQGTLVTVSS

SEQ ID NO: 75 - protein, 8 aa, synthetic construct
YYISRFYA

SEQ ID NO: 76 - protein, 7 aa, synthetic construct
ISSGGWT

SEQ ID NO: 77 - protein, 111 aa, synthetic construct
EVQLVESGGGLVQPGGSLRLSCAASYFISRFYAVGWYRQAPGKQRELVARISSGGWTYYADSVKGRFTISIDNSKNTLYLQMNSLRAEDTAVYYCNARNLWGQGTLVTVSS

SEQ ID NO: 78 - protein, 8 aa, synthetic construct
YFISRFYA

SEQ ID NO: 79 - protein, 111 aa, synthetic construct
EVQLVESGGGLVQPGGSLRLSCAASHYISRFYAVGWYRQAPGKQRELVARISSGGWTYYADSVKGRFTISIDNSKNTLYLQMNSLRAEDTAVYYCNARNLWGQGTLVTVSS

SEQ ID NO: 80 - protein, 8 aa, synthetic construct
HYISRFYA

SEQ ID NO: 81 - protein, 111 aa, synthetic construct
EVQLVESGGGLVQPGGSLRLSCAASHSISRFYAIGWYRQAPGKQRELVARISSMGRTYYADSVKGRFTISIDNSKNTLYLQMNSLRAEDTAVYYCNARNLWGQGTLVTVSS

SEQ ID NO: 82 - protein, 8 aa, synthetic construct
HSISRFYA

SEQ ID NO: 83 - protein, 7 aa, synthetic construct
ISSMGRT

SEQ ID NO: 84 - protein, 111 aa, synthetic construct
EVQLVESGGGLVQPGGSLRLSCAASGYISRFYAMGWYRQAPGKQRELVARISSGGWTYYADSVKGRFTISIDNSKNTLYLQMNSLRAEDTAVYYCNARNLWGQGTLVTVSS

SEQ ID NO: 85 - protein, 8 aa, synthetic construct
GYISRFYA

SEQ ID NO: 86 - protein, 111 aa, synthetic construct
EVQLVESGGGLVQPGGSLRLSCAASGYISRFYAMGWYRQAPGKQRELVARISSLGWTYYADSVKGRFTISIDNSKNTLYLQMNSLRAEDTAVYYCNARNLWGQGTLVTVSS

SEQ ID NO: 87 - protein, 7 aa, synthetic construct
ISSLGWT

SEQ ID NO: 88 - protein, 111 aa, synthetic construct
EVQLVESGGGLVQPGGSLRLSCAASGFISRFYAMGWYRQAPGKQRELVARISSMGWTYYADSVKGRFTISIDNSKNTLYLQMNSLRAEDTAVYYCNARNLWGQGTLVTVSS

SEQ ID NO: 89 - protein, 8 aa, synthetic construct
GFISRFYA

SEQ ID NO: 90 - protein, 7 aa, synthetic construct
ISSMGWT